European Patent Application EP 4 400 586 A1, published July 17, 2024. Title: Composition for Nucleic Acid Sequence Modification. Applicant: NATIONAL UNIVERSITY CORPORATION CHIBA UNIVERSITY. The sequence listing filed with the application follows.

SEQUENCE LISTING (13 sequences)

SEQ ID NO: 1 - protein, 360 aa, synthetic construct
  REGION 1..360: note = Synthetic
MHHHHHHSSGLVPRGSGMKETAAAKFERQHMDSPDLGTDDDDKAMADIGSQLVKSELEEKKSELRHKLKYVPHEYIELIEIARNSTQDRILEMKVMEFFMKVYGYRGKHLGGSRKPDGAIYTVGSPIDYGVIVDTKAYSGGYNLPIGQADEMQRYVEENQTRNKHINPNEWWKVYPSSVTEFKFLFVSGHFKGNYKAQLTRLNHITNCNGAVLSVEELLIGGEMIKAGTLTLEEVRRKFNNGEINFSGSETPGTSESATPESKDVVEIAVPENLVGAILGKGGKTLVEYQELTGARIQISKKGEFVPGTRNRKVTITGTPAATQAAQYLITQRITYEQGVRAANPQKVGSRADPKKKRKV

SEQ ID NO: 2 - RNA, 414 nt, synthetic construct
  misc_feature 1..414: note = Synthetic
  source 1..414: mol_type = other RNA
gggcgaattgggccctctagaaaacggccacaagttcagcgtgtccggcgagggcgagggcgatgccacctacggcaagctgaccctgaagttcatctgcaccaccggcaagctgcccgtgccctggcccaccctcgtgaccaccctgacctacggcgtgcagtgcttcagccgctaccccgaccacatgaagcagcacgacttcttcaagtccgccatgcccgaaggctacgtccaggagcgcaccatcttcttcaaggacgacggcaactacaagacccgcgccgaggtgaagttcgagggcgacacccactagtggatccgcagtctcatcatcattttcattttgttcgttagcacattgggcagtctcatcatcattttcattttgagatccgagctcggtaccaagct

SEQ ID NO: 3 - DNA, 4733 bp, synthetic construct
  misc_feature 1..4733: note = Synthetic
  source 1..4733: mol_type = other DNA
tagttattaatagtaatcaattacggggtcattagttcatagcccatatatggagttccgcgttacataacttacggtaaatggcccgcctggctgaccgcccaacgacccccgcccattgacgtcaataatgacgtatgttcccatagtaacgccaatagggactttccattgacgtcaatgggtggagtatttacggtaaactgcccacttggcagtacatcaagtgtatcatatgccaagtacgccccctattgacgtcaatgacggtaaatggcccgcctggcattatgcccagtacatgaccttatgggactttcctacttggcagtacatctacgtattagtcatcgctattaccatggtgatgcggttttggcagtacatcaatgggcgtggatagcggtttgactcacggggatttccaagtctccaccccattgacgtcaatgggagtttgttttggcaccaaaatcaacgggactttccaaaatgtcgtaacaactccgccccattgacgcaaatgggcggtaggcgtgtacggtgggaggtctatataagcagagctggtttagtgaaccgtcagatccgctagcgctaccggactcagatctcgagctcaagcttcgaattctgcagtcgacggtaccgcgggcccgggatccaccggtcgccaccatggtgagcaagggcgaggagctgttcaccggggtggtgcccatcctggtcgagctggacggcgacgtaaacggccacaagttcagcgtgtccggcgagggcgagggcgatgccacctacggcaagctgaccctgaagttcatctgcaccaccggcaagctgcccgtgccctggcccaccctcgtgaccaccctgacctacggcgtgcagtgcttcagccgctaccccgaccacatgaagcagcacgacttcttcaagtccgccatgcccgaaggctacgtccaggagcgcaccatcttcttcaaggacgacggcaactacaagacccgcgccgaggtgaagttcgagggcgacaccctggtgaaccgcatcgagctgaagggcatcgacttcaaggaggacggcaacatcctggggcacaagctggagtacaactacaacagccacaacgtctatatcatggccgacaagcagaagaacggcatcaaggtgaacttcaagatccgccacaacatcgaggacggcagcgtgcagctcgccgaccactaccagcagaacacccccatcggcgacggccccgtgctgctgcccgacaaccactacctgagcacccagtccgccctgagcaaagaccccaacgagaagcgcgatcacatggtcctgctggagttcgtgaccgccgccgggatcactctcggcatggacgagctgtacaagtaaagcggccgcgactctagatcataatcagccataccacatttgtagaggttttacttgctttaaaaaacctcccacacctccccctgaacctgaaacataaaatgaatgcaattgttgttgttaacttgtttattgcagcttataatggttacaaataaagcaatagcatcacaaatttcacaaataaagcatttttttcactgcattctagttgtggtttgtccaaactcatcaatgtatcttaaggcgtaaattgtaagcgttaatattttgttaaaattcgcgttaaatttttgttaaatcagctcattttttaaccaataggccgaaatcggcaaaatcccttataaatcaaaagaatagaccgagatagggttgagtgttgttccagtttggaacaagagtccactattaaagaacgtggactccaacgtcaaagggcgaaaaaccgtctatcagggcgatggcccactacgtgaaccatcaccctaatcaagttttttggggtcgaggtgccgtaaagcactaaatcggaaccctaaagggagcccccgatttagagcttgacggggaaagccggcgaacgtggcgagaaaggaagggaagaaagcgaaaggagcgggcgctagggcgctggcaagtgtagcggtcacgctgcgcgtaaccaccacacccgccgcgcttaatgcgccgctacagggcgcgtcaggtggcacttttcggggaaatgtgcgcggaacccctatttgtttatttttctaaatacattcaaatatgtatccgctcatgagacaataaccctgataaatgcttcaataatattgaaaaaggaagagtcctgaggcggaaagaaccagctgtggaatgtgtgtcagttagggtgtggaaagtccccaggctccccagcaggcagaagtatgcaaagcatgcatctcaattagtcagcaaccaggtgtggaaagtccccaggctccccagcaggcagaagtatgcaaagcatgcatctcaattagtcagcaaccatagtcccgcccctaactccgcccatcccgcccctaactccgcccagttccgcccattctccgccccatggctgactaattttttttatttatgcagaggccgaggccgcctcggcctctgagctattccagaagtagtgaggaggcttttttggaggcctaggcttttgcaaagatcgatcaagagacaggatgaggatcgtttcgcatgattgaacaagatggattgcacgcaggttctccggccgcttgggtggagaggctattcggctatgactgggcacaacagacaatcggctgctctgatgccgccgtgttccggctgtcagcgcaggggcgcccggttctttttgtcaagaccgacctgtccggtgccctgaatgaactgcaagacgaggcagcgcggctatcgtggctggccacgacgggcgttccttgcgcagctgtgctcgacgttgtcactgaagcgggaagggactggctgctattgggcgaagtgccggggcaggatctcctgtcatctcaccttgctcctgccgagaaagtatccatcatggctgatgcaatgcggcggctgcatacgcttgatccggctacctgcccattcgaccaccaagcgaaacatcgcatcgagcgagcacgtactcggatggaagccggtcttgtcgatcaggatgatctggacgaagagcatcaggggctcgcgccagccgaactgttcgccaggctcaaggcgagcatgcccgacggcgaggatctcgtcgtgacccatggcgatgcctgcttgccgaatatcatggtggaaaatggccgcttttctggattcatcgactgtggccggctgggtgtggcggaccgctatcaggacatagcgttggctacccgtgatattgctgaagagcttggcggcgaatgggctgaccgcttcctcgtgctttacggtatcgccgctcccgattcgcagcgcatcgccttctatcgccttcttgacgagttcttctgagcgggactctggggttcgaaatgaccgaccaagcgacgcccaacctgccatcacgagatttcgattccaccgccgccttctatgaaaggttgggcttcggaatcgttttccgggacgccggctggatgatcctccagcgcggggatctcatgctggagttcttcgcccaccctagggggaggctaactgaaacacggaaggagacaataccggaaggaacccgcgctatgacggcaataaaaagacagaataaaacgcacggtgttgggtcgtttgttcataaacgcggggttcggtcccagggctggcactctgtcgataccccaccgagaccccattggggccaatacgcccgcgtttcttccttttccccaccccaccccccaagttcgggtgaaggcccagggctcgcagccaacgtcggggcggcaggccctgccatagcctcaggttactcatatatactttagattgatttaaaacttcatttttaatttaaaaggatctaggtgaagatcctttttgataatctcatgaccaaaatcccttaacgtgagttttcgttccactgagcgtcagaccccgtagaaaagatcaaaggatcttcttgagatcctttttttctgcgcgtaatctgctgcttgcaaacaaaaaaaccaccgctaccagcggtggtttgtttgccggatcaagagctaccaactctttttccgaaggtaactggcttcagcagagcgcagataccaaatactgtccttctagtgtagccgtagttaggccaccacttcaagaactctgtagcaccgcctacatacctcgctctgctaatcctgttaccagtggctgctgccagtggcgataagtcgtgtcttaccgggttggactcaagacgatagttaccggataaggcgcagcggtcgggctgaacggggggttcgtgcacacagcccagcttggagcgaacgacctacaccgaactgagatacctacagcgtgagctatgagaaagcgccacgcttcccgaagggagaaaggcggacaggtatccggtaagcggcagggtcggaacaggagagcgcacgagggagcttccagggggaaacgcctggtatctttatagtcctgtcgggtttcgccacctctgacttgagcgtcgatttttgtgatgctcgtcaggggggcggagcctatggaaaaacgccagcaacgcggcctttttacggttcctggccttttgctggccttttgctcacatgttctttcctgcgttatcccctgattctgtggataaccgtattaccgccatgcat

SEQ ID NO: 4 - DNA, 32 bp, synthetic construct
  misc_feature 1..32: note = Synthetic
  source 1..32: mol_type = other DNA
gctctagaaaacggccacaagttcagcgtgtc

SEQ ID NO: 5 - DNA, 32 bp, synthetic construct
  misc_feature 1..32: note = Synthetic
  source 1..32: mol_type = other DNA
tgactagtgggtgtcgccctcgaacttcacct

SEQ ID NO: 6 - DNA, 60 bp, synthetic construct
  misc_feature 1..60: note = Synthetic
  source 1..60: mol_type = other DNA
tcggatccgcagtctcatcatcattttcattttgttcgttagcacattgggcagtctcat

SEQ ID NO: 7 - DNA, 60 bp, synthetic construct
  misc_feature 1..60: note = Synthetic
  source 1..60: mol_type = other DNA
gaagatctcaaaatgaaaatgatgatgagactgcccaatgtgctaacgaacaaaatgaaa

SEQ ID NO: 8 - RNA, 26 nt, synthetic construct
  misc_feature 1..26: note = Synthetic
  source 1..26: mol_type = other RNA
gcagtctcatcatcattttcattttg

SEQ ID NO: 9 - DNA, 714 bp, synthetic construct
  misc_feature 1..714: note = Synthetic
  source 1..714: mol_type = other DNA
gtgagcaagggcgaggagctgttcaccggggtggtgcccatcctggtcgagctggacggcgacgtaaacggccacaagttcagcgtgtccggcgagggcgagggcgatgccacctacggcaagctgaccctgaagttcatctgcaccaccggcaagctgcccgtgccctggcccaccctcgtgaccaccctgacctacggcgtgcagtgcttcagccgctaccccgaccacatgaagcagcacgacttcttcaagtccgccatgcccgaaggctacgtccaggagcgcaccatcttcttcaaggacgacggcaactacaagacccgcgccgaggtgaagttcgagggcgacaccctggtgaaccgcatcgagctgaagggcatcgacttcaaggaggacggcaacatcctggggcacaagctggagtacaactacaacagccacaacgtctatatcatggccgacaagcagaagaacggcatcaaggtgaacttcaagatccgccacaacatcgaggacggcagcgtgcagctcgccgaccactaccagcagaacacccccatcggcgacggccccgtgctgctgcccgacaaccactacctgagcacccagtccgccctgagcaaagaccccaacgagaagcgcgatcacatggtcctgctggagttcgtgaccgccgccgggatcactctcggcatggacgagctgtacaag

SEQ ID NO: 10 - DNA, 21 bp, synthetic construct
  misc_feature 1..21: note = Synthetic
  source 1..21: mol_type = other DNA
gtgagcaagggcgaggagctg

SEQ ID NO: 11 - DNA, 22 bp, synthetic construct
  misc_feature 1..22: note = Synthetic
  source 1..22: mol_type = other DNA
cttgtacagctcgtccatgccg

SEQ ID NO: 12 - DNA, 20 bp, synthetic construct
  misc_feature 1..20: note = Synthetic
  source 1..20: mol_type = other DNA
tagcggctgaagcactgcac

SEQ ID NO: 13 - DNA, 23 bp, synthetic construct
  misc_feature 1..23: note = Synthetic
  source 1..23: mol_type = other DNA
acaagcagaagaacggcatcaag